European Patent Specification EP 3 393 255 B1, published February 28, 2024. Title: IMPROVED ENZYMATIC MODIFICATION OF WHEAT PHOSPHOLIPIDS IN BAKERY APPLICATIONS. Applicant: DuPont Nutrition Biosciences ApS SOE, Jorn Borch MIKKELSEN, Rene JORGENSEN, Tina. The sequence listing filed with the application follows.

SEQUENCE LISTING (6 sequences)

SEQ ID NO: 1 - protein, 279 aa, Fusarium heterosporum
  MISC_FEATURE: Phospholipase sn1;enzyme in POWERBAKE 4080 and POWERBAKE 4090 that acts on a polar lipid at the sn1 position (same as SEQ ID NO: 6 from US Patent 8,012,732; hereby incorporated by reference).  This enzyme is known to have both gala
EAEAAVGVTSTDFTNFKFYIQHGAAAYCNSGTAAGAKITCSNNGCPTIESNGVTVVASFTGSKTGIGGYVSTDSSRKEIVVAIRGSSNIRNWLTNLDFDQSDCSLVSGCGVHSGFQNAWAEISAQASAAVAKARKANPSFKVVATGHSLGGAVATLSAANLRAAGTPVDIYTYGAPRVGNAALSAFISNQAGGEFRVTHDKDPVPRLPPLIFGYRHTTPEYWLSGGGGDKVDYAISDVKVCEGAANLMCNGGTLGLDIDAHLHYFQATDACNAGGFSWR

SEQ ID NO: 2 - protein, 318 aa, Aeromonas salmonicida
  MISC_FEATURE: mature lipid acyltransferase (GCAT) derived from Aeromonas salmonicida (See US patent 9,175,271)
ADTRPAFSRIVMFGDSLSDTGKMYSKMRGYLPSSPPYYEGRFSNGPVWLEQLTKQFPGLTIANEAEGGATAVAYNKISWDPKYQVINNLDYEVTQFLQKDSFKPDDLVILWVGANDYLAYGWNTEQDAKRVRDAISDAANRMVLNGAKQILLFNLPDLGQNPSARSQKVVEAVSHVSAYHNKLLLNLARQLAPTGMVKLFEIDKQFAEMLRDPQNFGLSDVENPCYDGGYVWKPFATRSVSTDRQLSAFSPQERLAIAGNPLLAQAVASPMARRSASPLNCEGKMFWDQVHPTTVVHAALSERAATFIETQYEFLAHG

SEQ ID NO: 3 - protein, 124 aa, Aspergillus niger
  MISC_FEATURE: phospholipase A2 enzyme which acts on N-acyl phosphatidyl ethanolamine at the sn2 position found in MAXAPAL A2.
ALWQFRSMIKCAIPGSHPLMDFNNYGCYCGLGGSGTPVDELDRCCETHDNCYRDAKNLDSCKFLVDNPYTESYSYSCSNTEITCNSKNNACEAFICNCDRNAAICFSKAPYNKEHKNLDTKKYC

SEQ ID NO: 4 - protein, 167 aa, Myceliophthora thermophila
  MISC_FEATURE: phospholipase A2 enzyme (CRC08335) which acts on NAPE (N-acyl phosphatidyl ethanolamine) at the sn2 position
LPSIGKADAALVPRQSAIQITDQYLFDLTLPAFTAKRNARDPPSLIWDSDGCSSSPDNPFGFPFVPACHRHDFGYRNYKAQNRFTDAGKLSIDNNFKSDLYYQCESVSAKTACRALADVYYAAVRAFGGSTQDKRDDDLVKIYEEKVAIYNKAVEEAQAKGELWTLD

SEQ ID NO: 5 - DNA, 549 bp, Myceliophthora thermophila
  misc_feature: synthetic gene encoding a fungal phospholipase A2 enzyme (CRC08335) which acts on NAPE (N-acyl phosphatidyl ethanolamine) at the sn2 position
atgaagttcctgagcaccgcactttgccttgcatcttctgtcctggcacttccatctatcggtaaagcagacgcagcacttgttccacgtcaatctgcaatccagatcaccgaccagtaccttttcgaccttacccttccagcattcaccgcaaaacgtaacgcacgggatccaccatctcttatctgggattctgacggctgtagctcttctccagataacccattcggcttcccattcgttcctgcttgtcatcggcatgatttcggttaccggaactacaaggcacagaaccgtttcaccgacgcaggcaagctttctattgacaacaacttcaagagcgacctctactaccagtgcgagtctgtttctgcaaagacagcttgtcgggcacttgcagacgtctattacgcagcagttcgggcattcggaggttctacacaagataagcgggacgacgatctagttaagatctacgaagagaaggtcgccatctacaacaaggcagttgaagaggcacaagcaaagggcgagctttggacacttgat

SEQ ID NO: 6 - protein, 16 aa, Myceliophthora thermophila
  MISC_FEATURE: N-terminal signal peptide sequence per prediction
MKFLSTALCLASSVLA